European Patent Specification EP 3 955 930 B1, published November 6, 2024. Title: Methods for Predicting Neisseria Spp. Susceptibility to Cefixime. Applicant: The Regents of the University of California. The sequence listing filed with the application follows.

SEQUENCE LISTING (1 sequence)

SEQ ID NO: 1 - protein, 581 aa, Neisseria gonorrhoeae
MLIKSEYKPRMLPKEEQVKKPMTSNGRISFVLMAMAVLFACLIARGLYLQTVTYNFLKEQGDNRIVRTQALPATRGTVSDRNGAVLALSAPTESLFAVPKDMKEMPSAAQLERLSELVDVPVDVLRNKLEQKGKSFIWIKRQLDPKVAEEVKALGLENFVFEKELKRHYPMGNLFAHVIGFTDIDGKGQEGLELSLEDSLYGEDGAEVVLRDRQGNIVDSLDSPRNKAPQNGKDIILSLDQRIQTLAYEELNKAVEYHQAKAGTVVVLDARTGEILALANTPAYDPNRPGRADSEQRRNRAVTDMIEPGSAIKPFVIAKALDAGKTDLNERLNTQPYKIGPSPVRDTHVYPSLDVRGIMQKSSNVGTSKLSARFGAEEMYDFYHELGIGVRMHSGFPGETAGLLRNWRRWRPIEQATMSFGYGLQLSLLQLARAYTALTHDGVLLPLSFEKQAVAPQGKRIFKESTAREVRNLMVSVTEPGGTGTAGAVDGFDVGAKTGTARKFVNGRYADNKHVATFIGFAPAKNPRVIVAVTIDEPTAHGYYGGVVAGPPFKKIMGGSLNILGISPTKPLTAAAVKTPS